European Patent Specification EP 3 135 684 B1, published June 28, 2023. Title: Vaccine against streptococcal infections based on recombinant proteins. Applicant: Intervacc AB. The sequence listing filed with the application follows.

SEQUENCE LISTING (42 sequences)

SEQ ID NO: 1 - DNA, 33 bp, Artificial Sequence
  PCR primer
ggttggatccactaatcttagtgacaacatcac

SEQ ID NO: 2 - DNA, 32 bp, Artificial Sequence
  PCR primer
tccagagctccttgacagtaaagctggtatag

SEQ ID NO: 3 - DNA, 28 bp, Artificial Sequence
  PCR primer
agtggagctcttagacgcagcaacagtg

SEQ ID NO: 4 - DNA, 35 bp, Artificial Sequence
  PCR primer
caccctcgagttatttggctttgttgattaaggtc

SEQ ID NO: 5 - DNA, 29 bp, Artificial Sequence
  PCR primer
cgtagagctctcggaacccaatccatatc

SEQ ID NO: 6 - DNA, 29 bp, Artificial Sequence
  PCR primer
gaggtctagaaggaccttgtttgccattt

SEQ ID NO: 7 - DNA, 28 bp, Artificial Sequence
  PCR primer
agcatctagattatctggtccgccagga

SEQ ID NO: 8 - DNA, 30 bp, Artificial Sequence
  PCR primer
gaggctgcagtggacctcgggtaccgcctt

SEQ ID NO: 9 - DNA, 29 bp, Artificial Sequence
  PCR primer
agtactgcaggaccagccagcagcactaa

SEQ ID NO: 10 - DNA, 31 bp, Artificial Sequence
  PCR primer
tgcagagctctggcttttgggcagcttcttc

SEQ ID NO: 11 - DNA, 29 bp, Artificial Sequence
  PCR primer
catgggatccgcgactaccctagcaggac

SEQ ID NO: 12 - DNA, 31 bp, Artificial Sequence
  PCR primer
ctagccatgggtgcttaagcttttcaatctg

SEQ ID NO: 13 - DNA, 30 bp, Artificial Sequence
  PCR primer
agtaccatgggaaacgactactgctagtgc

SEQ ID NO: 14 - DNA, 31 bp, Artificial Sequence
  PCR primer
ctggctcgagttatttagcaaccaaggctgc

SEQ ID NO: 15 - DNA, 33 bp, Artificial Sequence
  PCR primer
tactggatccgacgattaccaaaggaatgctac

SEQ ID NO: 16 - DNA, 32 bp, Artificial Sequence
  PCR primer
tgatctcgagttagctcagtttctgccatatg

SEQ ID NO: 17 - DNA, 32 bp, Artificial Sequence
  PCR primer
gtcggatccgaggataaggttgtgcaaactag

SEQ ID NO: 18 - DNA, 32 bp, Artificial Sequence
  PCR primer
gcctctcgagggataagctagtctgtctttgg

SEQ ID NO: 19 - DNA, 33 bp, Artificial Sequence
  PCR primer
ggcagagctcgatacagcaagctataccatcac

SEQ ID NO: 20 - DNA, 35 bp, Artificial Sequence
  PCR primer
tatttctagaagttttataggtgaaaacgataacc

SEQ ID NO: 21 - DNA, 1961 bp, Artificial Sequence
  Recombinant gene fusion fragment
tctgttccaggggcccctgggatccgcgactaccctagcaggacaaacagaagtacgggctgataatatcttacgcttagatatgacagataaagaagcagttgaaaaattcgctaacgagcttaaaaatgaagtccataaaaactatcgtggtagtaatacttggcaaaagcttacccttatacttaatggttatcaaaaccttagagaacaaatagagaccgagctaaaaaatagtgaacaaaaagtaaaagagcttaatgataaggttaatagtgaaactcaaggaaaacaagagttacagaatcagcttgagaaagaaaaagaagagttagaaacactaaaaaaagagcttgaagctgagaaggctaaaggaactggagaaacagagaagcttcaaaaggaaattgaagcaaaaaatgcaatgatttctgacctacaaaaacagcttgaggaaactaagcaaagggttcaagagtttgaagctgaagtaggtaaattaatggccgaaaaggcagacctacaaacaaaattaaatgaacaagagcagcttaacgctaagcttcaaaaagaaattgaagacttaaaggctcagattgaaaagcttaagcacccatgggaaacgactactgctagtgcatttgaaaataatgggacaggtcaacatctgaactggcacatagatattccacaagaatatacagttgaattaggagaaccaattactatctcagatcttatgagtcaaattacggttactcgtaaaggtagtaatgggactgttaatgatggagatacttttgactttatttcgaatggagatggttcaagaggaattgatacccctggagtaaaaatatggtttgacttttacaatgctgcgggtacttcctttttaactgatgaaatgttagcttcgcctacatatgctgtaccggggggatcttatactattaaagcttgggtattctatgggaaaaatgataccaaaaagctcttcacatttaaactaaaaaattccaacagcaataaaactgagttaaggaagtcgttagaggaggctaagctaaaactcagccagcctgaaggaacgtattctgatgaatcactgcaagccttgcaatcagcggttactattggtaagacctatttaaacagtgaccctgatcaaaatacagtagatcaatctgttactactattgattccgctattactagtcttgttaatcttaatgctttaaatgaagctattaatcaagctacaccttttataacagatggcaaagagtatcctaaagaagcgtatgacggtcttgtgcaaaagcttgcagcggcagctaagcttcaaaattcatttggtccttcacaaggagatgttgataaggctgcgactgatttaacgcaagctcttacgacgcttaagactgctgtagcgcatgaagccttagatcaagccttggctaagctgttagagctttaccgagaaaatccaaatcttgctttgacatcagagtctttgaaggaattgtacaataaggccattgaagcagcaggtaccttctatagaactgttaacaaggataaagagagaaaagacatttccctttatgagctagagcgctacactacagaaacaaattcagttgttgatactattttaaaggtaaaggctgcgattgccgaagaaggaaaggcaaaattgcgttctgctttagaccaattaaatgctcttatcggagaaaatctagacctatctccatatacagcagcttctgctcaagcctatacagaccagctagctaaggctaaggaggtcgcagcagcgggtgagacagcttatgctcaggagacagaaccgacagctattactaacagcttggttaaggtgttaaatgctaagaaatccctctcagatgccaaggcagccttggttgctaaataactcgagcggccgcatcgtg

SEQ ID NO: 22 - protein, 649 aa, Artificial Sequence
  Recombinant fusion protein
LEVLFQGPLGSATTLAGQTEVRADNILRLDMTDKEAVEKFANELKNEVHKNYRGSNTWQKLTLILNGYQNLREQIETELKNSEQKVKELNDKVNSETQGKQELQNQLEKEKEELETLKKELEAEKAKGTGETEKLQKEIEAKNAMISDLQKQLEETKQRVQEFEAEVGKLMAEKADLQTKLNEQEQLNAKLQKEIEDLKAQIEKLKHPWETTTASAFENNGTGQHLNWHIDIPQEYTVELGEPITISDLMSQITVTRKGSNGTVNDGDTFDFISNGDGSRGIDTPGVKIWFDFYNAAGTSFLTDEMLASPTYAVPGGSYTIKAWVFYGKNDTKKLFTFKLKNSNSNKTELRKSLEEAKLKLSQPEGTYSDESLQALQSAVTIGKTYLNSDPDQNTVDQSVTTIDSAITSLVNLNALNEAINQATPFITDGKEYPKEAYDGLVQKLAAAAKLQNSFGPSQGDVDKAATDLTQALTTLKTAVAHEALDQALAKLLELYRENPNLALTSESLKELYNKAIEAAGTFYRTVNKDKERKDISLYELERYTTETNSVVDTILKVKAAIAEEGKAKLRSALDQLNALIGENLDLSPYTAASAQAYTDQLAKAKEVAAAGETAYAQETEPTAITNSLVKVLNAKKSLSDAKAALVAK

SEQ ID NO: 23 - DNA, 1962 bp, Artificial Sequence
  Recombinant gene fusion fragment
ctggaagttctgttccaggggcccctgggatccactaatcttagtgacaacatcacatcattgacggttgcttcttcatcactccgagatggagagagaacgacggtaaaggttgcgtttgatgacaaaaaacagaaaatcaaggcaggggatacgatagaggtcacctggcctacaagtggtaatgtctacattcagggctttaataaaaccataccgcttaatattagaggggtagatgttggtaccttggaggtcacgctagacaaggctgttttcacattcaatcaaaatattgaaacaatgcatgatgtctctggttggggagagtttgatattactgttagaaatgtgacacaaaccaccgctgaaacatcaggaacgaccacagtaaaggtaggcaatcgcactgctactatcactgttactaagcctgaggcaggcactggtaccagctcattttattataagactggtgatatgcagcccaatgatactgagcgtgtgagatggttcctgctgattaacaacaacaaggaatgggtggccaatactgttacagtcgaagacgatattcaaggtggtcaaaccttggatatgagcagctttgacatcaccgtatctggttatcgtaacgagcgcttcgttggggaaaacgctctgacagagtttcatacaacatttccaaattctgtcattacggcaacagataatcacattagtgtgcggttagatcaatatgatgcctcacaaaacactgtcaacattgcttataagacaaagataacggactttgaccaaaaagaatttgccaacaacagtaaaatctggtaccagattttatacaaggatcaggtatcgggtcaagagtcaaaccaccaagtagccaatatcaatgctaacggcggggttgatggcagtcgctataccagctttactgtcaaggagctctcggaacccaatccatatccagatgtgaggcgtttccttgatgagaagtacgatggagatgtggataaattatctaaacaacttcaaggttattttggtagtttaagagagtatatagagtttgaacttaaaaatggcaaacaaggtccttctagattatctggtccgccaggatacccacttactcgtgatttctcccgtaacttcctagaagaaaatactgcaaaatatttagatcaattaagagaacatctacagcacagatttagtgaacttgagagcttaacaagaaaattagagaaagaaggcggtacccgaggtccactgcaggaccagccagcagcactaaaatatccagaacctagagactattttcttcatactcgtgaaggtgatgttatttatgatgaggatataaaaagatattttgaggatttagaagcctatttaacagctagacttggtgggattgataaaaaagtagaagaagctgcccaaaagccagagctcttagacgcagcaacagtgttagagcctacaacagccttcattagagaagctgttagggaaatcaatcagctgagtgatgactacgctgacaatcaagagcttcaggctgttcttgctaatgctggagttgaggcacttgctgcagatactgttgatcaggctaaagcagctcttgacaaagcaaaggcagctgttgctggtgttcagcttgatgaagcaagacgtgaggcttacagaacaatcaatgccttaagtgatcagcacaaaagcgatcaaaaggttcagctagctctagttgctgcagcagctaaggtggcagatgctgcttcagttgatcaagtgaatgcagccattaatgatgctcatacagctattgcggacattacaggagcagccttgttggaggctaaagaagctgctatcaatgaactaaagcagtatggcattagtgattactatgtgaccttaatcaacaaagccaaataactcgagcggccgcat

SEQ ID NO: 24 - protein, 648 aa, Artificial Sequence
  Recombinant fusion protein
LEVLFQGPLGSTNLSDNITSLTVASSSLRDGERTTVKVAFDDKKQKIKAGDTIEVTWPTSGNVYIQGFNKTIPLNIRGVDVGTLEVTLDKAVFTFNQNIETMHDVSGWGEFDITVRNVTQTTAETSGTTTVKVGNRTATITVTKPEAGTGTSSFYYKTGDMQPNDTERVRWFLLINNNKEWVANTVTVEDDIQGGQTLDMSSFDITVSGYRNERFVGENALTEFHTTFPNSVITATDNHISVRLDQYDASQNTVNIAYKTKITDFDQKEFANNSKIWYQILYKDQVSGQESNHQVANINANGGVDGSRYTSFTVKELSEPNPYPDVRRFLDEKYDGDVDKLSKQLQGYFGSLREYIEFELKNGKQGPSRLSGPPGYPLTRDFSRNFLEENTAKYLDQLREHLQHRFSELESLTRKLEKEGGTRGPLQDQPAALKYPEPRDYFLHTREGDVIYDEDIKRYFEDLEAYLTARLGGIDKKVEEAAQKPELLDAATVLEPTTAFIREAVREINQLSDDYADNQELQAVLANAGVEALAADTVDQAKAALDKAKAAVAGVQLDEARREAYRTINALSDQHKSDQKVQLALVAAAAKVADAASVDQVNAAINDAHTAIADITGAALLEAKEAAINELKQYGISDYYVTLINKAK

SEQ ID NO: 25 - DNA, 996 bp, Streptococcus equi
ctggaagttctgttccaggggcccctgggatccgacgattaccaaaggaatgctacggaagcttatgccaaagaagtaccacatcagatcacttctgtatggaccaaaggtgttacaccactaacacccgagcagtttcgatataataacgaagatgtgatccatgcgccatatcttgctcatcaaggctggtacgatatcaccaaggccttcgatgggaaggataatctcttgtgtggcgcagcaacggcaggtaatatgctgcattggtggtttgatcaaaataaaacagagattgaagcctatttaagtaaacaccctgaaaagcaaaaaatcatttttaacaaccaagagctatttgatttgaaagctgctatcgataccaaggacagtcaaaccaatagtcagctttttaattattttagagataaagcctttccaaatctatcagcacgtcaactcggggttatgcctgatcttgttctagacatgtttatcaatggttactacttaaatgtgtttaaaacacagtctactgatgtcaatcgaccttatcaggacaaggacaaacgaggtggtattttcgatgctgttttcaccagaggagatcagacaacgctcttgacagctcgtcatgatttaaaaaataaaggactaaatgacatcagcaccattatcaagcaagaactgactgaaggaagagcccttgctttatcacatacctacgccaatgttagcattagccatgtgattaacttgtggggagctgattttaatgctgaaggaaaccttgaggccatctatgtcacagactcagatgctaatgcgtctattggtatgaaaaaatattttgtcggcattaatgctcatagacatgtcgccatttctgccaagaaaatagaaggagaaaacattggcgctcaagtattaggcttatttacgctttccagtggcaaggacatatggcagaaactgagctaactcgagcggccgcat

SEQ ID NO: 26 - protein, 326 aa, Streptococcus equi
LEVLFQGPLGSDDYQRNATEAYAKEVPHQITSVWTKGVTPLTPEQFRYNNEDVIHAPYLAHQGWYDITKAFDGKDNLLCGAATAGNMLHWWFDQNKTEIEAYLSKHPEKQKIIFNNQELFDLKAAIDTKDSQTNSQLFNYFRDKAFPNLSARQLGVMPDLVLDMFINGYYLNVFKTQSTDVNRPYQDKDKRGGIFDAVFTRGDQTTLLTARHDLKNKGLNDISTIIKQELTEGRALALSHTYANVSISHVINLWGADFNAEGNLEAIYVTDSDANASIGMKKYFVGINAHRHVAISAKKIEGENIGAQVLGLFTLSSGKDIWQKLS

SEQ ID NO: 27 - DNA, 1452 bp, Artificial Sequence
  Recombinant gene fusion fragment
ctggaagttctgttccaggggcccctgggatccactaatcttagtgacaacatcacatcattgacggttgcttcttcatcactccgagatggagagagaacgacggtaaaggttgcgtttgatgacaaaaaacagaaaatcaaggcaggggatacgatagaggtcacctggcctacaagtggtaatgtctacattcagggctttaataaaaccataccgcttaatattagaggggtagatgttggtaccttggaggtcacgctagacaaggctgttttcacattcaatcaaaatattgaaacaatgcatgatgtctctggttggggagagtttgatattactgttagaaatgtgacacaaaccaccgctgaaacatcaggaacgaccacagtaaaggtaggcaatcgcactgctactatcactgttactaagcctgaggcaggcactggtaccagctcattttattataagactggtgatatgcagcccaatgatactgagcgtgtgagatggttcctgctgattaacaacaacaaggaatgggtggccaatactgttacagtcgaagacgatattcaaggtggtcaaaccttggatatgagcagctttgacatcaccgtatctggttatcgtaacgagcgcttcgttggggaaaacgctctgacagagtttcatacaacatttccaaattctgtcattacggcaacagataatcacattagtgtgcggttagatcaatatgatgcctcacaaaacactgtcaacattgcttataagacaaagataacggactttgaccaaaaagaatttgccaacaacagtaaaatctggtaccagattttatacaaggatcaggtatcgggtcaagagtcaaaccaccaagtagccaatatcaatgctaacggcggggttgatggcagtcgctataccagctttactgtcaaggagctcttagacgcagcaacagtgttagagcctacaacagccttcattagagaagctgttagggaaatcaatcagctgagtgatgactacgctgacaatcaagagcttcaggctgttcttgctaatgctggagttgaggcacttgctgcagatactgttgatcaggctaaagcagctcttgacaaagcaaaggcagctgttgctggtgttcagcttgatgaagcaagacgtgaggcttacagaacaatcaatgccttaagtgatcagcacaaaagcgatcaaaaggttcagctagctctagttgctgcagcagctaaggtggcagatgctgcttcagttgatcaagtgaatgcagccattaatgatgctcatacagctattgcggacattacaggagcagccttgttggaggctaaagaagctgctatcaatgaactaaagcagtatggcattagtgattactatgtgaccttaatcaacaaagccaaataactcgagcggccgcat

SEQ ID NO: 28 - protein, 478 aa, Artificial Sequence
  Recombinant fusion protein
LEVLFQGPLGSTNLSDNITSLTVASSSLRDGERTTVKVAFDDKKQKIKAGDTIEVTWPTSGNVYIQGFNKTIPLNIRGVDVGTLEVTLDKAVFTFNQNIETMHDVSGWGEFDITVRNVTQTTAETSGTTTVKVGNRTATITVTKPEAGTGTSSFYYKTGDMQPNDTERVRWFLLINNNKEWVANTVTVEDDIQGGQTLDMSSFDITVSGYRNERFVGENALTEFHTTFPNSVITATDNHISVRLDQYDASQNTVNIAYKTKITDFDQKEFANNSKIWYQILYKDQVSGQESNHQVANINANGGVDGSRYTSFTVKELLDAATVLEPTTAFIREAVREINQLSDDYADNQELQAVLANAGVEALAADTVDQAKAALDKAKAAVAGVQLDEARREAYRTINALSDQHKSDQKVQLALVAAAAKVADAASVDQVNAAINDAHTAIADITGAALLEAKEAAINELKQYGISDYYVTLINKAK

SEQ ID NO: 29 - DNA, 2322 bp, Artificial Sequence
  Recombinant gene fusion fragment
ctggaagttctgttccaggggcccctgggatccgacgattaccaaaggaatgctacggaagcttatgccaaagaagtaccacatcagatcacttctgtatggaccaaaggtgttacaccactaacacccgagcagtttcgatataataacgaagatgtgatccatgcgccatatcttgctcatcaaggctggtacgatatcaccaaggccttcgatgggaaggataatctcttgtgtggcgcagcaacggcaggtaatatgctgcattggtggtttgatcaaaataaaacagagattgaagcctatttaagtaaacaccctgaaaagcaaaaaatcatttttaacaaccaagagctatttgatttgaaagctgctatcgataccaaggacagtcaaaccaatagtcagctttttaattattttagagataaagcctttccaaatctatcagcacgtcaactcggggttatgcctgatcttgttctagacatgtttatcaatggttactacttaaatgtgtttaaaacacagtctactgatgtcaatcgaccttatcaggacaaggacaaacgaggtggtattttcgatgctgttttcaccagaggagatcagacaacgctcttgacagctcgtcatgatttaaaaaataaaggactaaatgacatcagcaccattatcaagcaagaactgactgaaggaagagcccttgctttatcacatacctacgccaatgttagcattagccatgtgattaacttgtggggagctgattttaatgctgaaggaaaccttgaggccatctatgtcacagactcagatgctaatgcgtctattggtatgaaaaaatattttgtcggcattaatgctcatagacatgtcgccatttctgccaagaaaatagaaggagaaaacattggcgctcaagtattaggcttatttacgctttccagtggcaaggacatatggcagaaactgagcccatgggaaacgactactgctagtgcatttgaaaataatgggacaggtcaacatctgaactggcacatagatattccacaagaatatacagttgaattaggagaaccaattactatctcagatcttatgagtcaaattacggttactcgtaaaggtagtaatgggactgttaatgatggagatacttttgactttatttcgaatggagatggttcaagaggaattgatacccctggagtaaaaatatggtttgacttttacaatgctgcgggtacttcctttttaactgatgaaatgttagcttcgcctacatatgctgtaccggggggatcttatactattaaagcttgggtattctatgggaaaaatgataccaaaaagctcttcacatttaaactaaaaaattccaacagcaataaaactgagttaaggaagtcgttagaggaggctaagctaaaactcagccagcctgaaggaacgtattctgatgaatcactgcaagccttgcaatcagcggttactattggtaagacctatttaaacagtgaccctgatcaaaatacagtagatcaatctgttactactattgattccgctattactagtcttgttaatcttaatgctttaaatgaagctattaatcaagctacaccttttataacagatggcaaagagtatcctaaagaagcgtatgacggtcttgtgcaaaagcttgcagcggcagctaagcttcaaaattcatttggtccttcacaaggagatgttgataaggctgcgactgatttaacgcaagctcttacgacgcttaagactgctgtagcgcatgaagccttagatcaagccttggctaagctgttagagctttaccgagaaaatccaaatcttgctttgacatcagagtctttgaaggaattgtacaataaggccattgaagcagcaggtaccttctatagaactgttaacaaggataaagagagaaaagacatttccctttatgagctagagcgctacactacagaaacaaattcagttgttgatactattttaaaggtaaaggctgcgattgccgaagaaggaaaggcaaaattgcgttctgctttagaccaattaaatgctcttatcggagaaaatctagacctatctccatatacagcagcttctgctcaagcctatacagaccagctagctaaggctaaggaggtcgcagcagcgggtgagacagcttatgctcaggagacagaaccgacagctattactaacagcttggttaaggtgttaaatgctaagaaatccctctcagatgccaaggcagccttggttgctaaataactcgagcggccgcat

SEQ ID NO: 30 - protein, 768 aa, Artificial Sequence
  Recombinant fusion protein
LEVLFQGPLGSDDYQRNATEAYAKEVPHQITSVWTKGVTPLTPEQFRYNNEDVIHAPYLAHQGWYDITKAFDGKDNLLCGAATAGNMLHWWFDQNKTEIEAYLSKHPEKQKIIFNNQELFDLKAAIDTKDSQTNSQLFNYFRDKAFPNLSARQLGVMPDLVLDMFINGYYLNVFKTQSTDVNRPYQDKDKRGGIFDAVFTRGDQTTLLTARHDLKNKGLNDISTIIKQELTEGRALALSHTYANVSISHVINLWGADFNAEGNLEAIYVTDSDANASIGMKKYFVGINAHRHVAISAKKIEGENIGAQVLGLFTLSSGKDIWQKLSPWETTTASAFENNGTGQHLNWHIDIPQEYTVELGEPITISDLMSQITVTRKGSNGTVNDGDTFDFISNGDGSRGIDTPGVKIWFDFYNAAGTSFLTDEMLASPTYAVPGGSYTIKAWVFYGKNDTKKLFTFKLKNSNSNKTELRKSLEEAKLKLSQPEGTYSDESLQALQSAVTIGKTYLNSDPDQNTVDQSVTTIDSAITSLVNLNALNEAINQATPFITDGKEYPKEAYDGLVQKLAAAAKLQNSFGPSQGDVDKAATDLTQALTTLKTAVAHEALDQALAKLLELYRENPNLALTSESLKELYNKAIEAAGTFYRTVNKDKERKDISLYELERYTTETNSVVDTILKVKAAIAEEGKAKLRSALDQLNALIGENLDLSPYTAASAQAYTDQLAKAKEVAAAGETAYAQETEPTAITNSLVKVLNAKKSLSDAKAALVAK

SEQ ID NO: 31 - DNA, 3004 bp, Streptococcus equi
ctggaagttctgttccaggggcccctgggatccgaggataaggttgtgcaaactagtccatcagtctctgctattgatgacctacattacctgtcggaaaacagtaaaaaagaatttaaggaggggttatcaaaggcaggagaagtacctgaaaagctaaaggatattttatccaaggcacagcaggcagataagcaggcaaaggttcttgcagaaatgaaggttcctgaaaaaatagccatgaagcctttaaaggggcctctttatggtggctattttaggacttggcatgataaaacatcagatccggctgaaaaggataaggttaattctatgggagaattgcctaaggaggttgacttagcctttgttttccatgattggaccaaggattatagctttttctggcaagaattggcgaccaagcatgtgccaacgctgaacaagcagggaacacgtgtgattcgtaccattccatggcggttccttgcaggcggtgatcatagtggtattgctgaagatacgcaaaaatacccaaatactccagagggaaataaggccttggcaaaggctattgtagatgaatacgtttataaatataatcttgatggtttagatgttgatattgagcgggatagcattccaaaagtaaatggaaaagagagtaacgaaaatattcagcgctctattgctgtttttgaagaaattggcaagcttattgggccaaagggcgctgacaagtcacgtttgttcattatggatagcacctacatggctgacaagaacccattgattgagcgcggtgcccaatatattgatttgctgcttgtgcaggtttatggcactcaaggtgagaagggagattgggatccagtcgctagaaaacctgaaaagacaatggaggaacgttgggaatcgtatagcaaatacattcgtcctgagcagtacatggttggtttttctttctatgaggaatatgcgggcagtggtaacctctggtatgatattaatgagaggaaagatgatcataatccgttaaattcagagatagctggtactcgtgctgagcgttatgcaaaatggcagcctaagacaggtggtgtcaagggagggattttctcttatgcgattgatcgcgatggtgtagcgcatcaacctaaaaaagtctcagatgatgagaaaagaactaacaaggctataaaggatataacagatggtattgtcaaatcagattataaggtttctaaggccttgaagaaggttatggaaaatgacaaatcctatgagctgattgatcagaaagattttccagacaaggctttgcgagaagcagttattgcacaggttggaagcagaagaggggatttagagcggttcaatggaaccctgcgcttagacaatccggatatcaagagtttagaaggcctgaataagcttaaaaaactagctaagctagagctaatcggtctatcacaaatcacaaagctggatagcttagtcctacctgcaaatgctaagccgaccaaggatacgctggccaatgttcttgaagcctacgacagcgctaagaaggaagagactaaggcgattccacaggtggctctgaccatttctggtctaactggcttgaaggaattaaatcttgctggctttgatcgtgatagcttggctggaattgacgcagctagcctaacctctcttgaaaaggtggatctctctagtaataagctggacttagcagctggtacggaaaatcgtcagattcttgataccatgctggcaacagtgactaagcatggcggtgttagcgaaaagacgtttgtatttgatcatcaaaagcctactggtctttatcctgatacttatggcactaagagccttcagttaccagtagcaaatgatacaattgatttgcaggctaagcttttatttggaacagttaccaatcagggcacgctaatcaatagcgaagctgactataaggcttatcaggagcaggaaatagcaggtcaccgttttgttgattcaagctatgattacaaagcctttgcagtgacctacaaggactataagatcaaggtgactgactcaaccttaggtgtcactgatcacaaggacttatccactagcaaggaggagacctacaaggttgaattctttagccctactaatagcactaagcctgtgcatgaggctaaggttgtcgttggtgcggaaaaaaccatgatggttaacctagcagagggagcaactgtgattggtggtgatgcagatccaacaaatgcaaaaaaagtgtttgatggtttgctcaataatgatacaacaattctgtcaactagcaataaagcttctatcatttttgaacttaaagagcctggcttagtcaagtattggcgtttctttaatgacagcaaaattagtaaagctgactgtattaaggaggccaagcttgaagcctttgttggccatcttgaagctggctcaaaggtaaaggatagcttggaaaaatcatcaaaatgggtaacagtttcagattattcaggagaggaccaagagtttagccagccgttaaacaacattggtgccaaatattggagaataacagttgatactaagggaggacgttacaattggccatcacttcctgagcttcaaatcattggttatcaattaccggctgcggatcttgtgatggcaatgctagctactgcagaggagctatctcagcaaaaagacaagttctctcaagagcagcttaaggagctcgaagtcaaaatagctgccttaaaggctgctttagatagtaagatgtttaatgccgatgctattaacgctagtactgctgatctgaaggcttatgttgataagcttttagctgatagaactgatcaggaaaaagtagctaaagcagctaaagttgagcagcctgtggctactgacataaaagaaaatactgagccagaaaatccaaagacagactagcttatccctcgagcggccgcat

SEQ ID NO: 32 - protein, 993 aa, Streptococcus equi
LEVLFQGPLGSEDKVVQTSPSVSAIDDLHYLSENSKKEFKEGLSKAGEVPEKLKDILSKAQQADKQAKVLAEMKVPEKIAMKPLKGPLYGGYFRTWHDKTSDPAEKDKVNSMGELPKEVDLAFVFHDWTKDYSFFWQELATKHVPTLNKQGTRVIRTIPWRFLAGGDHSGIAEDTQKYPNTPEGNKALAKAIVDEYVYKYNLDGLDVDIERDSIPKVNGKESNENIQRSIAVFEEIGKLIGPKGADKSRLFIMDSTYMADKNPLIERGAQYIDLLLVQVYGTQGEKGDWDPVARKPEKTMEERWESYSKYIRPEQYMVGFSFYEEYAGSGNLWYDINERKDDHNPLNSEIAGTRAERYAKWQPKTGGVKGGIFSYAIDRDGVAHQPKKVSDDEKRTNKAIKDITDGIVKSDYKVSKALKKVMENDKSYELIDQKDFPDKALREAVIAQVGSRRGDLERFNGTLRLDNPDIKSLEGLNKLKKLAKLELIGLSQITKLDSLVLPANAKPTKDTLANVLEAYDSAKKEETKAIPQVALTISGLTGLKELNLAGFDRDSLAGIDAASLTSLEKVDLSSNKLDLAAGTENRQILDTMLATVTKHGGVSEKTFVFDHQKPTGLYPDTYGTKSLQLPVANDTIDLQAKLLFGTVTNQGTLINSEADYKAYQEQEIAGHRFVDSSYDYKAFAVTYKDYKIKVTDSTLGVTDHKDLSTSKEETYKVEFFSPTNSTKPVHEAKVVVGAEKTMMVNLAEGATVIGGDADPTNAKKVFDGLLNNDTTILSTSNKASIIFELKEPGLVKYWRFFNDSKISKADCIKEAKLEAFVGHLEAGSKVKDSLEKSSKWVTVSDYSGEDQEFSQPLNNIGAKYWRITVDTKGGRYNWPSLPELQIIGYQLPAADLVMAMLATAEELSQQKDKFSQEQLKELEVKIAALKAALDSKMFNADAINASTADLKAYVDKLLADRTDQEKVAKAAKVEQPVATDIKENTEPENPKTD

SEQ ID NO: 33 - DNA, 2715 bp, Artificial Sequence
  Recombinant gene fusion fragment
ctggaagttctgttccaggggcccctgggatccactaatcttagtgacaacatcacatcattgacggttgcttcttcatcactccgagatggagagagaacgacggtaaaggttgcgtttgatgacaaaaaacagaaaatcaaggcaggggatacgatagaggtcacctggcctacaagtggtaatgtctacattcagggctttaataaaaccataccgcttaatattagaggggtagatgttggtaccttggaggtcacgctagacaaggctgttttcacattcaatcaaaatattgaaacaatgcatgatgtctctggttggggagagtttgatattactgttagaaatgtgacacaaaccaccgctgaaacatcaggaacgaccacagtaaaggtaggcaatcgcactgctactatcactgttactaagcctgaggcaggcactggtaccagctcattttattataagactggtgatatgcagcccaatgatactgagcgtgtgagatggttcctgctgattaacaacaacaaggaatgggtggccaatactgttacagtcgaagacgatattcaaggtggtcaaaccttggatatgagcagctttgacatcaccgtatctggttatcgtaacgagcgcttcgttggggaaaacgctctgacagagtttcatacaacatttccaaattctgtcattacggcaacagataatcacattagtgtgcggttagatcaatatgatgcctcacaaaacactgtcaacattgcttataagacaaagataacggactttgaccaaaaagaatttgccaacaacagtaaaatctggtaccagattttatacaaggatcaggtatcgggtcaagagtcaaaccaccaagtagccaatatcaatgctaacggcggggttgatggcagtcgctataccagctttactgtcaaggagctcgatacagcaagctataccatcactgttgagggagctacagcaggtcacacctatgaggcttatcagattttcaagggtgacttgtttgacagtaccctatcaaacatcacatggggaggtggtgttacaccttttgaatttgatggttcaaaagacgctgctaagattgcagagggattgaaggaagcaaatgcagctgcctttgccaaggaagcaggtaagcacttgacagcaaccattgcaggaacaggaacacatgcaatcaccgttaacgaggctggctactacctcatcaaggacaaaaatgattctcaaacaggcaagcatgacgcctacacctcatttgtcctgaaggttgttaaaaacaccagcttcaaaccaaaatctgctatcccaacagtccttaaaaaggtcaaggaccgtaatgacaagacaggtcttgagacaggctggcaagattcagctgactatgacaaaaatgacaaggtgccattccagctaaccgcaaccctaccgtcaaattacgatgcctttcaagaatactaccttgaatttgtagataccttatcaaaagggctaagctacaacaaagacgccaaggtctatgtggttaatggagatactcgtcaagatattactaattcatttacagttagtgaagatggttcatcttttaaaatcaataacctaaaggctgttcagggagtaacaataacagctaccagtaagatcgttgtcgaatacactgctaccctcaatgaccaagcggccatcggcaaaaaaggaaatccaaacgaagttgctttgaaatactcaaacgatccaaacgctcttggaaaaggagaggagtctccaaaaggggagacaccaaaagacaaggttatcgttttcacctataaaacttctagattatctggtccgccaggatacccacttactcgtgatttctcccgtaacttcctagaagaaaatactgcaaaatatttagatcaattaagagaacatctacagcacagatttagtgaacttgagagcttaacaagaaaattagagaaagaaggcggtacccgaggtccactgcaggaccagccagcagcactaaaatatccagaacctagagactattttcttcatactcgtgaaggtgatgttatttatgatgaggatataaaaagatattttgaggatttagaagcctatttaacagctagacttggtgggattgataaaaaagtagaagaagctgcccaaaagccagagctcttagacgcagcaacagtgttagagcctacaacagccttcattagagaagctgttagggaaatcaatcagctgagtgatgactacgctgacaatcaagagcttcaggctgttcttgctaatgctggagttgaggcacttgctgcagatactgttgatcaggctaaagcagctcttgacaaagcaaaggcagctgttgctggtgttcagcttgatgaagcaagacgtgaggcttacagaacaatcaatgccttaagtgatcagcacaaaagcgatcaaaaggttcagctagctctagttgctgcagcagctaaggtggcagatgctgcttcagttgatcaagtgaatgcagccattaatgatgctcatacagctattgcggacattacaggagcagccttgttggaggctaaagaagctgctatcaatgaactaaagcagtatggcattagtgattactatgtgaccttaatcaacaaagccaaataactcgagcggccgcat

SEQ ID NO: 34 - protein, 899 aa, Artificial Sequence
  Recombinant fusion protein
LEVLFQGPLGSTNLSDNITSLTVASSSLRDGERTTVKVAFDDKKQKIKAGDTIEVTWPTSGNVYIQGFNKTIPLNIRGVDVGTLEVTLDKAVFTFNQNIETMHDVSGWGEFDITVRNVTQTTAETSGTTTVKVGNRTATITVTKPEAGTGTSSFYYKTGDMQPNDTERVRWFLLINNNKEWVANTVTVEDDIQGGQTLDMSSFDITVSGYRNERFVGENALTEFHTTFPNSVITATDNHISVRLDQYDASQNTVNIAYKTKITDFDQKEFANNSKIWYQILYKDQVSGQESNHQVANINANGGVDGSRYTSFTVKELDTASYTITVEGATAGHTYEAYQIFKGDLFDSTLSNITWGGGVTPFEFDGSKDAAKIAEGLKEANAAAFAKEAGKHLTATIAGTGTHAITVNEAGYYLIKDKNDSQTGKHDAYTSFVLKVVKNTSFKPKSAIPTVLKKVKDRNDKTGLETGWQDSADYDKNDKVPFQLTATLPSNYDAFQEYYLEFVDTLSKGLSYNKDAKVYVVNGDTRQDITNSFTVSEDGSSFKINNLKAVQGVTITATSKIVVEYTATLNDQAAIGKKGNPNEVALKYSNDPNALGKGEESPKGETPKDKVIVFTYKTSRLSGPPGYPLTRDFSRNFLEENTAKYLDQLREHLQHRFSELESLTRKLEKEGGTRGPLQDQPAALKYPEPRDYFLHTREGDVIYDEDIKRYFEDLEAYLTARLGGIDKKVEEAAQKPELLDAATVLEPTTAFIREAVREINQLSDDYADNQELQAVLANAGVEALAADTVDQAKAALDKAKAAVAGVQLDEARREAYRTINALSDQHKSDQKVQLALVAAAAKVADAASVDQVNAAINDAHTAIADITGAALLEAKEAAINELKQYGISDYYVTLINKAK

SEQ ID NO: 35 - DNA, 28 bp, Artificial Sequence
  PCR primer
gcatccatggatacagcaagctatacca

SEQ ID NO: 36 - DNA, 31 bp, Artificial Sequence
  PCR primer
caattattttttcccagataggagctcagct

SEQ ID NO: 37 - DNA, 1283 bp, Streptococcus equi
ccatggatacagcaagctataccatcactgttgagggagctacagcaggtcacacctatgaggcttatcagattttcaagggtgacttgtttgacagtaccctatcaaacatcacatggggaggtggtgttacaccttttgaatttgatggttcaaaagacgctgctaagattgcagagggattgaaggaagcaaatgcagctgcctttgccaaggaagcaggtaagcacttgacagcaaccattgcaggaacaggaacacatgcaatcaccgttaacgaggctggctactacctcatcaaggacaaaaatgattctcaaacaggcaagcatgacgcctacacctcatttgtcctgaaggttgttaaaaacaccagcttcaaaccaaaatctgctatcccaacagtccttaaaaaggtcaaggaccgtaatgacaagacaggtcttgagacaggctggcaagattcagctgactatgacaaaaatgacaaggtgccattccagctaaccgcaaccctaccgtcaaattacgatgcctttcaagaatactaccttgaatttgtagataccttatcaaaagggctaagctacaacaaagacgccaaggtctatgtggttaatggagatactcgtcaagatattactaattcatttacagttagtgaagatggttcatcttttaaaatcaataacctaaaggctgttcagggagtaacaataacagctaccagtaagatcgttgtcgaatacactgctaccctcaatgaccaagcggccatcggcaaaaaaggaaatccaaacgaagttgctttgaaatactcaaacgatccaaacgctcttggaaaaggagaggagtctccaaaaggggagacaccaaaagacaaggttatcgttttcacctataaaactatcatcaataaggttgatcaagatcaaaaagccctaaaaggtgcaggctttaccctttataagctggtcaaaggtgataatggcgaggaaaaatatcaaatagtccaagaaattaaagcaggggatacaactagctttgagtttgttggacttgacgctggtgattacaagctcagcgaaacaacaacacctggcggttacaacactattgcagatgtcatgttcagcattgtagcgcagcatgaaaccgagtcagacgatcctcagttgactagcctaaccgttgacaaagcaactggcttcactgctgatacagaagctggtaccgtatccgcaactattgttaataaaaggtctatcctcgagcccgggtgc

SEQ ID NO: 38 - protein, 426 aa, Streptococcus equi
MDTASYTITVEGATAGHTYEAYQIFKGDLFDSTLSNITWGGGVTPFEFDGSKDAAKIAEGLKEANAAAFAKEAGKHLTATIAGTGTHAITVNEAGYYLIKDKNDSQTGKHDAYTSFVLKVVKNTSFKPKSAIPTVLKKVKDRNDKTGLETGWQDSADYDKNDKVPFQLTATLPSNYDAFQEYYLEFVDTLSKGLSYNKDAKVYVVNGDTRQDITNSFTVSEDGSSFKINNLKAVQGVTITATSKIVVEYTATLNDQAAIGKKGNPNEVALKYSNDPNALGKGEESPKGETPKDKVIVFTYKTIINKVDQDQKALKGAGFTLYKLVKGDNGEEKYQIVQEIKAGDTTSFEFVGLDAGDYKLSETTTPGGYNTIADVMFSIVAQHETESDDPQLTSLTVDKATGFTADTEAGTVSATIVNKRSILEPG

SEQ ID NO: 39 - DNA, 29 bp, Artificial Sequence
  PCR primer
gcagccatggagagtctgacgagtgttga

SEQ ID NO: 40 - DNA, 31 bp, Artificial Sequence
  PCR primer
tcacctcgagtcctagctcaccgtcataagc

SEQ ID NO: 41 - DNA, 1301 bp, Streptococcus equi
ccatggagagtctgacgagtgttgagcctgctgatggtgcggtcatggtcaagtcagaggctgctgaccaaggctcaaatgagctaccagaagctactgacattagtgatattgctggtatttctgatgtgactaaggtgtcagctgctgtcaatgctgatactgtcaaggaagttcagccagtagctgtacctcttgtagaggatcaggcgcatgaggaaactacagaccagtctcagccttcatcatcgatagtgtctgttacgacagacagctctctagagacaccagaagctacaagctcagaggagccgatagcggagcagaccttgcggctgcatttcaagaccctgccagctcaagacctatcctcgcttggtctttgggtgtgggacgatgttgagacaccatctgatcagctgggaggctggccgactggggctaccaattttagtctagcgaagacagatgactatggctattacatggacgttaagctttcagccaatcaagccaataaggttagctttttgatcaataacactaagggagacaatctgacgggcgatcgaaccatagaccttctcagccctaagatgaatgaggtctggattgatggccaggagctgtcttactatcggccgctggctcagggctatatccgtatcaattattatcgcagtgatggccattatgacaacaaatcgctctggctttggggaagtgctgatgcgtcaatgactagtcagcagggcgcttggccagatggtattgattttaagcaggtcggtcgatatggtgcttatatagatgtcaagctagctgataccaatgagctaggctttctcttgctagatgagcgtcagacaggtgacgctgttaaaattcagcccaatgattatatttttaaagatttaaagaatcacacccaaattttcttgaaagacgaggatccaaccatttatacgaacccttattttgttaatacagttagattaatcggtgctcagcaggtcagcccaagcagtattgaggcgagctttacgactctagcagatgtggataaggaaagccttttaaaagaattaaaaatcagcactgacagtaaggaagcagttgctattactgatatcaccttagatgaaaagactcataaggctgtcatcacaggtgattttagtcaagcagtggccacttatacggtgacctttcatcatgagagcttccaggctaggccaaattggcaatacaaggatagcctgtatgcttatgacggtgagctaggactcgagcccgggtgc

SEQ ID NO: 42 - protein, 432 aa, Streptococcus equi
MESLTSVEPADGAVMVKSEAADQGSNELPEATDISDIAGISDVTKVSAAVNADTVKEVQPVAVPLVEDQAHEETTDQSQPSSSIVSVTTDSSLETPEATSSEEPIAEQTLRLHFKTLPAQDLSSLGLWVWDDVETPSDQLGGWPTGATNFSLAKTDDYGYYMDVKLSANQANKVSFLINNTKGDNLTGDRTIDLLSPKMNEVWIDGQELSYYRPLAQGYIRINYYRSDGHYDNKSLWLWGSADASMTSQQGAWPDGIDFKQVGRYGAYIDVKLADTNELGFLLLDERQTGDAVKIQPNDYIFKDLKNHTQIFLKDEDPTIYTNPYFVNTVRLIGAQQVSPSSIEASFTTLADVDKESLLKELKISTDSKEAVAITDITLDEKTHKAVITGDFSQAVATYTVTFHHESFQARPNWQYKDSLYAYDGELGLEPG